European Patent Application EP 4 748 925 A1, published May 27, 2026. Title: 신규한 리보스 포스페이트 디포스포키나제 변이체 및 이를 이용한 L-아미노산 생산 방법. Applicant: CJ CheilJedang Corporation. Application KR. The sequence listing filed with the application follows.

SEQUENCE LISTING (52 sequences)

SEQ ID NO: 1 - protein, 317 aa, unidentified
MSNQYGDKNLKIFSLNSNPELAKEIADIVGVQLGKCSVTRFSDGEVQINIEESIRGCDCYIIQSTSDPVNEHIMELLIMVDALKRASAKTINIVIPYYGYARQDRKARSREPITAKLFANLLETAGATRVIALDLHAPQIQGFFDIPIDHLMGVPILGEYFEGKNLEDIVIVSPDHGGVTRARKLADRLKAPIAIIDKRRPRPNVAEVMNIVGNIEGKTAILIDDIIDTAGTITLAANALVENGAKEVYACCTHPVLSGPAVERINNSTIKELVVTNSIKLPEEKKIERFKQLSVGPLLAEAIIRVHEQQSVSYLFS

SEQ ID NO: 2 - DNA, 954 bp, unidentified
  source 1..954: mol_type = genomic DNA
atgtctaatcaatacggagataagaatttaaagattttttctttgaattcgaatccagagcttgcaaaagaaatcgcagatatagttggagttcaattagggaaatgttctgtcacaagatttagtgacggggaagtccaaattaatatcgaagaaagtattcgcggatgtgattgttacatcatccagtctacaagtgaccccgttaacgagcatattatggaactgctgattatggtagatgcgttaaaacgcgcttctgcaaaaacgattaacattgttattccttattacggttatgcgcgtcaagacagaaaagcaagatcccgtgagccaatcacagctaaacttttcgctaacctgcttgaaacagccggtgcgactcgtgtgattgcacttgacctgcatgcgccgcaaattcaaggattctttgatataccgattgaccacttaatgggtgttccgattttaggagaatattttgaaggcaaaaatcttgaagatatcgtcattgtttcaccagaccatggcggtgtgacacgtgcccgcaaactggctgaccgactaaaagcgccaattgcgattatcgataaacgccgtccgcgtccaaacgtggcggaagtcatgaatattgtaggtaacatcgaagggaagactgctatcctcatcgatgacattattgatactgcaggtacgattacacttgctgctaatgcgctcgttgaaaacggagcgaaagaagtatatgcatgctgtacacaccctgtactatcaggccctgcggttgaacggattaataattcaacaattaaagagcttgttgtgacaaacagcatcaagcttcctgaagaaaagaaaattgaacgctttaagcagctttcagtcggaccgcttctggccgaagcgattattcgcgttcatgagcagcaatcagtcagctatctgttcagctaa

SEQ ID NO: 3 - DNA, 38 bp, synthetic construct
  source 1..38: mol_type = other DNA
aacgacggccagtgaattctcgttggccattacctcat

SEQ ID NO: 4 - DNA, 45 bp, synthetic construct
  source 1..45: mol_type = other DNA
ctgtttagtactaaaccggaagggccttatctgccacacccacaa

SEQ ID NO: 5 - DNA, 45 bp, synthetic construct
  source 1..45: mol_type = other DNA
cggtttagtactaaacaggaagagcctaaaaacggaagagccact

SEQ ID NO: 6 - DNA, 39 bp, synthetic construct
  source 1..39: mol_type = other DNA
ttgcatgcctgcaggtcgacggaagactatccaaggtgg

SEQ ID NO: 7 - DNA, 40 bp, synthetic construct
  source 1..40: mol_type = other DNA
taaggcccttccggtttagtagaaacatcccagcgctact

SEQ ID NO: 8 - DNA, 40 bp, synthetic construct
  source 1..40: mol_type = other DNA
tctccgtattgattagacatgagtgtttcctttcgttggg

SEQ ID NO: 9 - DNA, 40 bp, synthetic construct
  source 1..40: mol_type = other DNA
cccaacgaaaggaaacactcatgtctaatcaatacggaga

SEQ ID NO: 10 - DNA, 40 bp, synthetic construct
  source 1..40: mol_type = other DNA
ttaggctcttcctgtttagtttagctgaacagatagctga

SEQ ID NO: 11 - DNA, 16 bp, synthetic construct
  source 1..16: mol_type = other DNA
ccagcgactaagcttg

SEQ ID NO: 12 - DNA, 16 bp, synthetic construct
  source 1..16: mol_type = other DNA
aagccatccaagcagc

SEQ ID NO: 13 - DNA, 18 bp, synthetic construct
  source 1..18: mol_type = other DNA
gttcggcttggattatgg

SEQ ID NO: 14 - DNA, 18 bp, synthetic construct
  source 1..18: mol_type = other DNA
catcaacaacagccttca

SEQ ID NO: 15 - protein, 317 aa, synthetic construct
MSNQYGDKNLKIFSLNSNPELAKEIADIVGVQLGKCSVTRFSDGEVQINIEESIRGCDCYIIQSTSDPVNEHIMELLIMVDALKRASAKTINIVIPYYGYARQDRKARSREPITAKLFANLLETAGATRVIALDLHAPQIQGFFDIPIDHLMGVPILGEYFEGKNLEDIVIVSPDHGGVTRARKLADRLKAPIAIIDKRRPRPNVAEVMNIVGNIEGKTAILIDDIIDTAGTITLAANVLVENGAKEVYACCTHPVLSGPAVERINNSTIKELVVTNSIKLPEEKKIERFKQLSVGPLLAEAIIRVHEQQSVSYLFS

SEQ ID NO: 16 - protein, 317 aa, synthetic construct
MSNQYGDKNLKIFSLNSNPELAKEIADIVGVQLGKCSVTRFSDGEVQINIEESIRGCDCYIIQSTSDPVNEHIMELLIMVDALKRASAKTINIVIPYYGYARQDRKARSREPITAKLFANLLETAGATRVIALDLHAPQIQGFFDIPIDHLMGVPILGEYFEGKNLEDIVIVSPDHGGVTRARKLADRLKAPIAIIDKRRPRPNVAEVMNIVGNIEGKTAILIDDIIDTAGTITLAANPLVENGAKEVYACCTHPVLSGPAVERINNSTIKELVVTNSIKLPEEKKIERFKQLSVGPLLAEAIIRVHEQQSVSYLFS

SEQ ID NO: 17 - protein, 317 aa, synthetic construct
MSNQYGDKNLKIFSLNSNPELAKEIADIVGVQLGKCSVTRFSDGEVQINIEESIRGCDCYIIQSTSDPVNEHIMELLIMVDALKRASAKTINIVIPYYGYARQDRKARSREPITAKLFANLLETAGATRVIALDLHAPQIQGFFDIPIDHLMGVPILGEYFEGKNLEDIVIVSPDHGGVTRARKLADRLKAPIAIIDKRRPRPNVAEVMNIVGNIEGKTAILIDDIIDTAGTITLAANNLVENGAKEVYACCTHPVLSGPAVERINNSTIKELVVTNSIKLPEEKKIERFKQLSVGPLLAEAIIRVHEQQSVSYLFS

SEQ ID NO: 18 - protein, 317 aa, synthetic construct
MSNQYGDKNLKIFSLNSNPELAKEIADIVGVQLGKCSVTRFSDGEVQINIEESIRGCDCYIIQSTSDPVNEHIMELLIMVDALKRASAKTINIVIPYYGYARQDRKARSREPITAKLFANLLETAGATRVIALDLHAPQIQGFFDIPIDHLMGVPILGEYFEGKNLEDIVIVSPDHGGVTRARKLADRLKAPIAIIDKRRPRPNVAEVMNIVGNIEGKTAILIDDIIDTAGTITLAANMLVENGAKEVYACCTHPVLSGPAVERINNSTIKELVVTNSIKLPEEKKIERFKQLSVGPLLAEAIIRVHEQQSVSYLFS

SEQ ID NO: 19 - protein, 317 aa, synthetic construct
MSNQYGDKNLKIFSLNSNPELAKEIADIVGVQLGKCSVTRFSDGEVQINIEESIRGCDCYIIQSTSDPVNEHIMELLIMVDALKRASAKTINIVIPYYGYARQDRKARSREPITAKLFANLLETAGATRVIALDLHAPQIQGFFDIPIDHLMGVPILGEYFEGKNLEDIVIVSPDHGGVTRARKLADRLKAPIAIIDKRRPRPNVAEVMNIVGNIEGKTAILIDDIIDTAGTITLAANGLVENGAKEVYACCTHPVLSGPAVERINNSTIKELVVTNSIKLPEEKKIERFKQLSVGPLLAEAIIRVHEQQSVSYLFS

SEQ ID NO: 20 - protein, 317 aa, synthetic construct
MSNQYGDKNLKIFSLNSNPELAKEIADIVGVQLGKCSVTRFSDGEVQINIEESIRGCDCYIIQSTSDPVNEHIMELLIMVDALKRASAKTINIVIPYYGYARQDRKARSREPITAKLFANLLETAGATRVIALDLHAPQIQGFFDIPIDHLMGVPILGEYFEGKNLEDIVIVSPDHGGVTRARKLADRLKAPIAIIDKRRPRPNVAEVMNIVGNIEGKTAILIDDIIDTAGTITLAANYLVENGAKEVYACCTHPVLSGPAVERINNSTIKELVVTNSIKLPEEKKIERFKQLSVGPLLAEAIIRVHEQQSVSYLFS

SEQ ID NO: 21 - DNA, 35 bp, synthetic construct
  source 1..35: mol_type = other DNA
cttgctgctaatgtgctcgttgaaaacggagcgaa

SEQ ID NO: 22 - DNA, 35 bp, synthetic construct
  source 1..35: mol_type = other DNA
ctccgttttcaacgagcacattagcagcaagtgta

SEQ ID NO: 23 - DNA, 35 bp, synthetic construct
  source 1..35: mol_type = other DNA
cttgctgctaatccactcgttgaaaacggagcgaa

SEQ ID NO: 24 - DNA, 35 bp, synthetic construct
  source 1..35: mol_type = other DNA
ctccgttttcaacgagtggattagcagcaagtgta

SEQ ID NO: 25 - DNA, 35 bp, synthetic construct
  source 1..35: mol_type = other DNA
cttgctgctaataacctcgttgaaaacggagcgaa

SEQ ID NO: 26 - DNA, 35 bp, synthetic construct
  source 1..35: mol_type = other DNA
ctccgttttcaacgaggttattagcagcaagtgta

SEQ ID NO: 27 - DNA, 35 bp, synthetic construct
  source 1..35: mol_type = other DNA
cttgctgctaatatgctcgttgaaaacggagcgaa

SEQ ID NO: 28 - DNA, 35 bp, synthetic construct
  source 1..35: mol_type = other DNA
ctccgttttcaacgagcatattagcagcaagtgta

SEQ ID NO: 29 - DNA, 35 bp, synthetic construct
  source 1..35: mol_type = other DNA
cttgctgctaatggcctcgttgaaaacggagcgaa

SEQ ID NO: 30 - DNA, 35 bp, synthetic construct
  source 1..35: mol_type = other DNA
ctccgttttcaacgaggccattagcagcaagtgta

SEQ ID NO: 31 - DNA, 35 bp, synthetic construct
  source 1..35: mol_type = other DNA
cttgctgctaattacctcgttgaaaacggagcgaa

SEQ ID NO: 32 - DNA, 35 bp, synthetic construct
  source 1..35: mol_type = other DNA
ctccgttttcaacgaggtaattagcagcaagtgta

SEQ ID NO: 33 - DNA, 18 bp, synthetic construct
  source 1..18: mol_type = other DNA
gttcggcttggattatgg

SEQ ID NO: 34 - DNA, 18 bp, synthetic construct
  source 1..18: mol_type = other DNA
catcaacaacagccttca

SEQ ID NO: 35 - DNA, 37 bp, synthetic construct
  source 1..37: mol_type = other DNA
gaattcgagctcggtacccgacacatccgcaccggac

SEQ ID NO: 36 - DNA, 45 bp, synthetic construct
  source 1..45: mol_type = other DNA
gacttttcttcttacgctgctgagtactgcttgcttagagtcctg

SEQ ID NO: 37 - DNA, 45 bp, synthetic construct
  source 1..45: mol_type = other DNA
atcaggactctaagcaagcagtactcagcagcgtaagaagaaaag

SEQ ID NO: 38 - DNA, 45 bp, synthetic construct
  source 1..45: mol_type = other DNA
tgcaggtcgactctagaggatccccttgatgactcttagggctag

SEQ ID NO: 39 - DNA, 50 bp, synthetic construct
  source 1..50: mol_type = other DNA
cacaattttggaggattacaagaacatgtctaatcaatacggagataaga

SEQ ID NO: 40 - DNA, 50 bp, synthetic construct
  source 1..50: mol_type = other DNA
attgacttttcttcttacgctgctgagtttagctgaacagatagctgact

SEQ ID NO: 41 - DNA, 40 bp, synthetic construct
  source 1..40: mol_type = other DNA
gaatcaggactctaagcaagcagtgccgtgcgtggcgagt

SEQ ID NO: 42 - DNA, 50 bp, synthetic construct
  source 1..50: mol_type = other DNA
tcttatctccgtattgattagacatgttcttgtaatcctccaaaattgtg

SEQ ID NO: 43 - DNA, 22 bp, synthetic construct
  source 1..22: mol_type = other DNA
acatccttcttattcagctcag

SEQ ID NO: 44 - DNA, 20 bp, synthetic construct
  source 1..20: mol_type = other DNA
tggttttagtccgatcgagg

SEQ ID NO: 45 - DNA, 35 bp, synthetic construct; identical to SEQ ID NO: 21
  source 1..35: mol_type = other DNA

SEQ ID NO: 46 - DNA, 35 bp, synthetic construct; identical to SEQ ID NO: 22
  source 1..35: mol_type = other DNA

SEQ ID NO: 47 - DNA, 954 bp, synthetic construct
  source 1..954: mol_type = other DNA
atgtctaatcaatacggagataagaatttaaagattttttctttgaattcgaatccagagcttgcaaaagaaatcgcagatatagttggagttcaattagggaaatgttctgtcacaagatttagtgacggggaagtccaaattaatatcgaagaaagtattcgcggatgtgactgttatatcatccagtctacaagtgaccccgttaacgagcatattatggaactgttgattatggtagatgcgttaaaacgcgcttctgcaaaaacgattaacattgtgattccttattacggttatgcgcgtcaagacagaaaagcaagatcccgtgagccaatcacagcaaaactttttgctaacctgcttgaaacagccggtgcgactcgtgtgattgcacttgacctgcatgcgccgcaaattcaaggattctttgatataccgattgaccacttaatgggtgttccgattttaggagaatattttgagggcaaaaaccttgaagatatcgtcattgtttccccagaccacggcggcgtgacacgcgcccgcaaactggctgaccgactaaaagcaccgattgcgattatcgataaacgccgtccgcgtccaaacgtggcggaagtcatgaatattgtaggtaatatcgaagggaagaccgctatccttatcgatgacattatcgatactgcaggtaccattacacttgctgctaatgtgctcgttgaaaacggagcgaaagaagtatatgcatgctgtacacaccctgtactgtcaggcccagctgttgaacggattaataattcaacaattaaagagcttgttgtgacaaacagcatcaagcttcctgaagaaaagaaaattgaacggtttaagcagctttcagtcggaccgcttttggctgaagcgattattcgcgttcatgagcagcaatcagtcagctatctgttcagctaa

SEQ ID NO: 48 - DNA, 954 bp, synthetic construct
  source 1..954: mol_type = other DNA
atgtctaatcaatacggagataagaatttaaagattttttctttgaattcgaatccagagcttgcaaaagaaatcgcagatatagttggagttcaattagggaaatgttctgtcacaagatttagtgacggggaagtccaaattaatatcgaagaaagtattcgcggatgtgactgttatatcatccagtctacaagtgaccccgttaacgagcatattatggaactgttgattatggtagatgcgttaaaacgcgcttctgcaaaaacgattaacattgtgattccttattacggttatgcgcgtcaagacagaaaagcaagatcccgtgagccaatcacagcaaaactttttgctaacctgcttgaaacagccggtgcgactcgtgtgattgcacttgacctgcatgcgccgcaaattcaaggattctttgatataccgattgaccacttaatgggtgttccgattttaggagaatattttgagggcaaaaaccttgaagatatcgtcattgtttccccagaccacggcggcgtgacacgcgcccgcaaactggctgaccgactaaaagcaccgattgcgattatcgataaacgccgtccgcgtccaaacgtggcggaagtcatgaatattgtaggtaatatcgaagggaagaccgctatccttatcgatgacattatcgatactgcaggtaccattacacttgctgctaatccactcgttgaaaacggagcgaaagaagtatatgcatgctgtacacaccctgtactgtcaggcccagctgttgaacggattaataattcaacaattaaagagcttgttgtgacaaacagcatcaagcttcctgaagaaaagaaaattgaacggtttaagcagctttcagtcggaccgcttttggctgaagcgattattcgcgttcatgagcagcaatcagtcagctatctgttcagctaa

SEQ ID NO: 49 - DNA, 954 bp, synthetic construct
  source 1..954: mol_type = other DNA
atgtctaatcaatacggagataagaatttaaagattttttctttgaattcgaatccagagcttgcaaaagaaatcgcagatatagttggagttcaattagggaaatgttctgtcacaagatttagtgacggggaagtccaaattaatatcgaagaaagtattcgcggatgtgactgttatatcatccagtctacaagtgaccccgttaacgagcatattatggaactgttgattatggtagatgcgttaaaacgcgcttctgcaaaaacgattaacattgtgattccttattacggttatgcgcgtcaagacagaaaagcaagatcccgtgagccaatcacagcaaaactttttgctaacctgcttgaaacagccggtgcgactcgtgtgattgcacttgacctgcatgcgccgcaaattcaaggattctttgatataccgattgaccacttaatgggtgttccgattttaggagaatattttgagggcaaaaaccttgaagatatcgtcattgtttccccagaccacggcggcgtgacacgcgcccgcaaactggctgaccgactaaaagcaccgattgcgattatcgataaacgccgtccgcgtccaaacgtggcggaagtcatgaatattgtaggtaatatcgaagggaagaccgctatccttatcgatgacattatcgatactgcaggtaccattacacttgctgctaataacctcgttgaaaacggagcgaaagaagtatatgcatgctgtacacaccctgtactgtcaggcccagctgttgaacggattaataattcaacaattaaagagcttgttgtgacaaacagcatcaagcttcctgaagaaaagaaaattgaacggtttaagcagctttcagtcggaccgcttttggctgaagcgattattcgcgttcatgagcagcaatcagtcagctatctgttcagctaa

SEQ ID NO: 50 - DNA, 954 bp, synthetic construct
  source 1..954: mol_type = other DNA
atgtctaatcaatacggagataagaatttaaagattttttctttgaattcgaatccagagcttgcaaaagaaatcgcagatatagttggagttcaattagggaaatgttctgtcacaagatttagtgacggggaagtccaaattaatatcgaagaaagtattcgcggatgtgactgttatatcatccagtctacaagtgaccccgttaacgagcatattatggaactgttgattatggtagatgcgttaaaacgcgcttctgcaaaaacgattaacattgtgattccttattacggttatgcgcgtcaagacagaaaagcaagatcccgtgagccaatcacagcaaaactttttgctaacctgcttgaaacagccggtgcgactcgtgtgattgcacttgacctgcatgcgccgcaaattcaaggattctttgatataccgattgaccacttaatgggtgttccgattttaggagaatattttgagggcaaaaaccttgaagatatcgtcattgtttccccagaccacggcggcgtgacacgcgcccgcaaactggctgaccgactaaaagcaccgattgcgattatcgataaacgccgtccgcgtccaaacgtggcggaagtcatgaatattgtaggtaatatcgaagggaagaccgctatccttatcgatgacattatcgatactgcaggtaccattacacttgctgctaatatgctcgttgaaaacggagcgaaagaagtatatgcatgctgtacacaccctgtactgtcaggcccagctgttgaacggattaataattcaacaattaaagagcttgttgtgacaaacagcatcaagcttcctgaagaaaagaaaattgaacggtttaagcagctttcagtcggaccgcttttggctgaagcgattattcgcgttcatgagcagcaatcagtcagctatctgttcagctaa

SEQ ID NO: 51 - DNA, 954 bp, synthetic construct
  source 1..954: mol_type = other DNA
atgtctaatcaatacggagataagaatttaaagattttttctttgaattcgaatccagagcttgcaaaagaaatcgcagatatagttggagttcaattagggaaatgttctgtcacaagatttagtgacggggaagtccaaattaatatcgaagaaagtattcgcggatgtgactgttatatcatccagtctacaagtgaccccgttaacgagcatattatggaactgttgattatggtagatgcgttaaaacgcgcttctgcaaaaacgattaacattgtgattccttattacggttatgcgcgtcaagacagaaaagcaagatcccgtgagccaatcacagcaaaactttttgctaacctgcttgaaacagccggtgcgactcgtgtgattgcacttgacctgcatgcgccgcaaattcaaggattctttgatataccgattgaccacttaatgggtgttccgattttaggagaatattttgagggcaaaaaccttgaagatatcgtcattgtttccccagaccacggcggcgtgacacgcgcccgcaaactggctgaccgactaaaagcaccgattgcgattatcgataaacgccgtccgcgtccaaacgtggcggaagtcatgaatattgtaggtaatatcgaagggaagaccgctatccttatcgatgacattatcgatactgcaggtaccattacacttgctgctaatggcctcgttgaaaacggagcgaaagaagtatatgcatgctgtacacaccctgtactgtcaggcccagctgttgaacggattaataattcaacaattaaagagcttgttgtgacaaacagcatcaagcttcctgaagaaaagaaaattgaacggtttaagcagctttcagtcggaccgcttttggctgaagcgattattcgcgttcatgagcagcaatcagtcagctatctgttcagctaa

SEQ ID NO: 52 - DNA, 954 bp, synthetic construct
  source 1..954: mol_type = other DNA
atgtctaatcaatacggagataagaatttaaagattttttctttgaattcgaatccagagcttgcaaaagaaatcgcagatatagttggagttcaattagggaaatgttctgtcacaagatttagtgacggggaagtccaaattaatatcgaagaaagtattcgcggatgtgactgttatatcatccagtctacaagtgaccccgttaacgagcatattatggaactgttgattatggtagatgcgttaaaacgcgcttctgcaaaaacgattaacattgtgattccttattacggttatgcgcgtcaagacagaaaagcaagatcccgtgagccaatcacagcaaaactttttgctaacctgcttgaaacagccggtgcgactcgtgtgattgcacttgacctgcatgcgccgcaaattcaaggattctttgatataccgattgaccacttaatgggtgttccgattttaggagaatattttgagggcaaaaaccttgaagatatcgtcattgtttccccagaccacggcggcgtgacacgcgcccgcaaactggctgaccgactaaaagcaccgattgcgattatcgataaacgccgtccgcgtccaaacgtggcggaagtcatgaatattgtaggtaatatcgaagggaagaccgctatccttatcgatgacattatcgatactgcaggtaccattacacttgctgctaattacctcgttgaaaacggagcgaaagaagtatatgcatgctgtacacaccctgtactgtcaggcccagctgttgaacggattaataattcaacaattaaagagcttgttgtgacaaacagcatcaagcttcctgaagaaaagaaaattgaacggtttaagcagctttcagtcggaccgcttttggctgaagcgattattcgcgttcatgagcagcaatcagtcagctatctgttcagctaa